European Patent Application EP 4 534 545 A1, published April 9, 2025. Title: Novel peptide and used thereof. Applicant: ZINCURE CORP. Application KR. The sequence listing filed with the application follows.

SEQUENCE LISTING (15 sequences)

SEQ ID NO: 1 - protein, 5 aa, synthetic construct
  REGION 1..5: note = ZC303
  VARIANT 3: note = D-form
  VARIANT 4: note = D-form
HGVSG

SEQ ID NO: 2 - protein, 5 aa, synthetic construct
  REGION 1..5: note = ZC304
  VARIANT 1: note = D-form
HGVSG

SEQ ID NO: 3 - protein, 6 aa, synthetic construct
  REGION 1..6: note = ZC305
  VARIANT 1: note = D-form
  VARIANT 3: note = D-form
  VARIANT 4: note = D-form
  VARIANT 6: note = D-form
HGVSGD

SEQ ID NO: 4 - protein, 6 aa, synthetic construct
  REGION 1..6: note = ZC306
  VARIANT 1: note = D-form
  VARIANT 3: note = D-form
  VARIANT 4: note = D-form
  VARIANT 6: note = D-form
HGVSGS

SEQ ID NO: 5 - protein, 6 aa, synthetic construct
  REGION 1..6: note = ZC307
  VARIANT 1: note = D-form
  VARIANT 3: note = D-form
  VARIANT 4: note = D-form
  VARIANT 6: note = D-form
HGVSGN

SEQ ID NO: 6 - protein, 6 aa, synthetic construct
  REGION 1..6: note = ZC308
  VARIANT 1: note = D-form
  VARIANT 3: note = D-form
  VARIANT 4: note = D-form
  VARIANT 6: note = D-form
HGVSGY

SEQ ID NO: 7 - protein, 6 aa, synthetic construct
  REGION 1..6: note = ZC309
  VARIANT 1: note = D-form
  VARIANT 4: note = D-form
  VARIANT 6: note = D-form
HGVSGH

SEQ ID NO: 8 - protein, 6 aa, synthetic construct
  REGION 1..6: note = ZC310
  VARIANT 1: note = D-form
  VARIANT 3: note = D-form
  VARIANT 6: note = D-form
HGVSGH

SEQ ID NO: 9 - protein, 5 aa, synthetic construct
  REGION 1..5: note = ZC311
  VARIANT 1: note = D-form
  VARIANT 4: note = D-form
HGQHG

SEQ ID NO: 10 - protein, 5 aa, synthetic construct
  REGION 1..5: note = ZC312
  VARIANT 1: note = D-form
  VARIANT 3: note = D-form
  VARIANT 4: note = D-form
HGQVG

SEQ ID NO: 11 - protein, 4 aa, synthetic construct
  REGION 1..4: note = ZC313
  VARIANT 1: note = D-form
  VARIANT 3: note = D-form
HGVG

SEQ ID NO: 12 - protein, 5 aa, synthetic construct
  REGION 1..5: note = ZC314
  VARIANT 1: note = D-form
  VARIANT 3: note = D-form
HGHGL

SEQ ID NO: 13 - protein, 5 aa, synthetic construct
  REGION 1..5: note = ZC315
  VARIANT 1: note = D-form
  VARIANT 3: note = D-form
  VARIANT 4: note = D-form
HGVTG

SEQ ID NO: 14 - protein, 5 aa, synthetic construct
  REGION 1..5: note = ZC316
  VARIANT 1: note = D-form
  VARIANT 3: note = D-form
  VARIANT 4: note = D-form
HGVCG

SEQ ID NO: 15 - protein, 5 aa, synthetic construct
  REGION 1..5: note = ZC317
  VARIANT 1: note = D-form
  VARIANT 3: note = D-form
  VARIANT 4: note = D-form
HGVWG